European Patent Specification EP 3 215 182 B1, published January 4, 2023. Title: COMBINATION IMMUNOTHERAPY. Applicant: Dubinett, et al.,. The sequence listing filed with the application follows.

SEQUENCE LISTING (4 sequences)

SEQ ID NO: 1 - protein, 134 aa, Homo sapiens
MAQSLALSLLILVLAFGIPRTQGSDGGAQDCCLKYSQRKIPAKVVRSYRKQEPSLGCSIPAILFLPRKRSQAELCADPKELWVQQLMQHLDKTPSPQKPAQGCRKDRGASKTGKKGKGSKGCKRTERSQTPKGP

SEQ ID NO: 2 - protein, 133 aa, Murine
MAQMMTLSLLSLDLALCIPWTQGSDGGGQDCCLKYSQKKIPYSIVRGYRKQEPSLGCPIPAILFLPRKHSKPELCANPEEGWVQNLMRRLDQPPAPGKQSPGCRKNRGTSKSGKKGKGSKGCKRTEQTQPSRG

SEQ ID NO: 3 - DNA, 23 bp, Murine
tggaccttctaggtcttgaaagg

SEQ ID NO: 4 - DNA, 24 bp, Murine
aggcattccaccactgctcccatt